European Patent Application EP 4 653 538 A1, published November 26, 2025. Title: Method for producing nucleic acid-transfected cells and method for producing useful substance. Applicant: FUJIFILM Corporation. The sequence listing filed with the application follows.

SEQUENCE LISTING (3 sequences)

SEQ ID NO: 1 - DNA, 6073 bp, synthetic construct
  misc_feature 1..6073: note = plasmid
  source 1..6073: mol_type = other DNA
gatccacgggtggcatccctgtgacccctccccagtgcctctcctggccctggaagttgccactccagtgcccaccagccttgtcctaataaaattaagttgcatcattttgtctgactaggtgtccttctataatattatggggtggaggggggtggtatggagcaaggggcaagttgggaagacaacctgtagggcctgcggggtctattgggaaccaagctggagtgcagtggcacaatcttggctcactgcaatctccgcctcctgggttcaagcgattctcctgcctcagcctcccgagttgttgggattccaggcatgcatgaccaggctcagctaatttttgtttttttggtagagacggggtttcaccatattggccaggctggtctccaactcctaatctcaggtgatctacccaccttggcctcccaaattgctgggattacaggcgtgaaccactgctcccttccctgtccttatcgatagatctaggaacccctagtgatggagttggccactccctctctgcgcgctcgctcgctcactgaggccgggcgaccaaaggtcgcccgacgcccgggctttgcccgggcggcctcagtgagcgagcgagcgcgcagctgcctgcaggcagcttggcactggccgtcgttttacaacgtcgtgactgggaaaaccctggcgttacccaacttaatcgccttgcagcacatccccctttcgccagctggcgtaatagcgaagaggcccgcaccgatcgcccttcccaacagttgcgcagcctgaatggcgaatggcgcctgatgcggtattttctccttacgcatctgtgcggtatttcacaccgcatacgtcaaagcaaccatagtacgcgccctgtagcggcgcattaagcgcggcgggtgtggtggttacgcgcagcgtgaccgctacacttgccagcgccctagcgcccgctcctttcgctttcttcccttcctttctcgccacgttcgccggctttccccgtcaagctctaaatcgggggctccctttagggttccgatttagtgctttacggcacctcgaccccaaaaaacttgatttgggtgatggttcacgtagtgggccatcgccctgatagacggtttttcgccctttgacgttggagtccacgttctttaatagtggactcttgttccaaactggaacaacactcaaccctatctcgggctattcttttgatttataagggattttgccgatttcggcctattggttaaaaaatgagctgatttaacaaaaatttaacgcgaattttaacaaaatattaacgtttacaattttatggtgcactctcagtacaatctgctctgatgccgcatagttaagccagccccgacacccgccaacacccgctgacgcgccctgacgggcttgtctgctcccggcatccgcttacagacaagctgtgaccgtctccgggagctgcatgtgtcagaggttttcaccgtcatcaccgaaacgcgcgagacgaaagggcctcgtgatacgcctatttttataggttaatgtcatgataataatggtttcttagacgtcaggtggcacttttcggggaaatgtgcgcggaacccctatttgtttatttttctaaatacattcaaatatgtatccgctcatgagacaataaccctgataaatgcttcaataatattgaaaaaggaagagtatgagtattcaacatttccgtgtcgcccttattcccttttttgcggcattttgccttcctgtttttgctcacccagaaacgctggtgaaagtaaaagatgctgaagatcagttgggtgcacgagtgggttacatcgaactggatctcaacagcggtaagatccttgagagttttcgccccgaagaacgttttccaatgatgagcacttttaaagttctgctatgtggcgcggtattatcccgtattgacgccgggcaagagcaactcggtcgccgcatacactattctcagaatgacttggttgagtactcaccagtcacagaaaagcatcttacggatggcatgacagtaagagaattatgcagtgctgccataaccatgagtgataacactgcggccaacttacttctgacaacgatcggaggaccgaaggagctaaccgcttttttgcacaacatgggggatcatgtaactcgccttgatcgttgggaaccggagctgaatgaagccataccaaacgacgagcgtgacaccacgatgcctgtagcaatggcaacaacgttgcgcaaactattaactggcgaactacttactctagcttcccggcaacaattaatagactggatggaggcggataaagttgcaggaccacttctgcgctcggcccttccggctggctggtttattgctgataaatctggagccggtgagcgtgggtctcgcggtatcattgcagcactggggccagatggtaagccctcccgtatcgtagttatctacacgacggggagtcaggcaactatggatgaacgaaatagacagatcgctgagataggtgcctcactgattaagcattggtaactgtcagaccaagtttactcatatatactttagattgatttaaaacttcatttttaatttaaaaggatctaggtgaagatcctttttgataatctcatgaccaaaatcccttaacgtgagttttcgttccactgagcgtcagaccccgtagaaaagatcaaaggatcttcttgagatcctttttttctgcgcgtaatctgctgcttgcaaacaaaaaaaccaccgctaccagcggtggtttgtttgccggatcaagagctaccaactctttttccgaaggtaactggcttcagcagagcgcagataccaaatactgttcttctagtgtagccgtagttaggccaccacttcaagaactctgtagcaccgcctacatacctcgctctgctaatcctgttaccagtggctgctgccagtggcgataagtcgtgtcttaccgggttggactcaagacgatagttaccggataaggcgcagcggtcgggctgaacggggggttcgtgcacacagcccagcttggagcgaacgacctacaccgaactgagatacctacagcgtgagctatgagaaagcgccacgcttcccgaagggagaaaggcggacaggtatccggtaagcggcagggtcggaacaggagagcgcacgagggagcttccagggggaaacgcctggtatctttatagtcctgtcgggtttcgccacctctgacttgagcgtcgatttttgtgatgctcgtcaggggggcggagcctatggaaaaacgccagcaacgcggcctttttacggttcctggccttttgctggccttttgctcacatgttctttcctgcgttatcccctgattctgtggataaccgtattaccgcctttgagtgagctgataccgctcgccgcagccgaacgaccgagcgcagcgagtcagtgagcgaggaagcggaagagcgcccaatacgcaaaccgcctctccccgcgcgttggccgattcattaatgcagctggcacgacaggtttcccgactggaaagcgggcagtgagcgcaacgcaattaatgtgagttagctcactcattaggcaccccaggctttacactttatgcttccggctcgtatgttgtgtggaattgtgagcggataacaatttcacacaggaaacagctatgaccatgattacgaattgcctgcaggcagctgcgcgctcgctcgctcactgaggccgcccgggcaaagcccgggcgtcgggcgacctttggtcgcccggcctcagtgagcgagcgagcgcgcagagagggagtggccaactccatcactaggggttcctatcgatatcaagctttaatagtaatcaattacggggtcattagttcatagcccatatatggagttccgcgttacataacttacggtaaatggcccgcctggctgaccgcccaacgacccccgcccattgacgtcaataatgacgtatgttcccatagtaacgccaatagggactttccattgacgtcaatgggtggagtatttacggtaaactgcccacttggcagtacatcaagtgtatcatatgccaagtacgccccctattgacgtcaatgacggtaaatggcccgcctggcattatgcccagtacatgaccttatgggactttcctacttggcagtacatctacgtattagtcatcgctattaccatggtgatgcggttttggcagtacatcaatgggcgtggatagcggtttgactcacggggatttccaagtctccaccccattgacgtcaatgggagtttgttttggcaccaaaatcaacgggactttccaaaatgtcgtaacaactccgccccattgacgcaaatgggcggtaggcgtgtacggtgggaggtctatataagcagagctggtttagtggatatccttaagggcccagccggcctcgcgagaattctctagcaagctgtgaccggcgcctacgctagacgccaccatggagagcgacgagagcggcctgcccgccatggagatcgagtgccgcatcaccggcaccctgaacggcgtggagttcgagctggtgggcggcggagagggcacccccaagcagggccgcatgaccaacaagatgaagagcaccaaaggcgccctgaccttcagcccctacctgctgagccacgtgatgggctacggcttctaccacttcggcacctaccccagcggctacgagaaccccttcctgcacgccatcaacaacggcggctacaccaacacccgcatcgagaagtacgaggacggcggcgtgctgcacgtgagcttcagctaccgctacgaggccggccgcgtgatcggcgacttcaaggtggtgggcaccggcttccccgaggacagcgtgatcttcaccgacaagatcatccgcagcaacgccaccgtggagcacctgcaccccatgggcgataacgtgctggtgggcagcttcgcccgcaccttcagcctgcgcgacggcggctactacagcttcgtggtggacagccacatgcacttcaagagcgccatccaccccagcatcctgcagaacgggggccccatgttcgccttccgccgcgtggaggagctgcacagcaacaccgagctgggcatcgtggagtaccagcacgccttcaagacccccatcgccttcgccagatcccgcgctcagtcgtccaattctgccgtggacggcaccgccggacccggctccaccggatctcgcgagggcagaggaagtcttctaacatgcggtgacgtggaggagaatcccggccctatgaccgagtacaagcccacggtgcgcctcgccacccgcgacgacgtccccagggccgtacgcaccctcgccgccgcgttcgccgactaccccgccacgcgccacaccgtcgatccggaccgccacatcgagcgggtcaccgagctgcaagaactcttcctcacgcgcgtcgggctcgacatcggcaaggtgtgggtcgcggacgacggcgccgcggtggcggtctggaccacgccggagagcgtcgaagcgggggcggtgttcgccgagatcggcccgcgcatggccgagttgagcggttcccggctggccgcgcagcaacagatggaaggcctcctggcgccgcaccggcccaaggagcccgcgtggttcctggccaccgtcggcgtctcgcccgaccaccagggcaagggtctgggcagcgccgtcgtgctccccggagtggaggcggccgagcgcgccggggtgcccgccttcctggagacctccgcgccccgcaacctccccttctacgagcggctcggcttcaccgtcaccgccgacgtcgaggtgcccgaaggaccgcgcacctggtgcatgacccgcaagcccggtgcctgaaatcaacctctggattacaaaatttgtgaaagattgactggtattcttaactatgttgctccttttacgctatgtggatacgctgctttaatgcctttgtatcagtt

SEQ ID NO: 2 - DNA, 7294 bp, synthetic construct
  misc_feature 1..7294: note = plasmid
  source 1..7294: mol_type = other DNA
gcgcgccgatatcgttaacgccccgcgccggccgctctagaactagtggatcccccggaagatcagaagttcctattccgaagttcctattctctagaaagtataggaacttctgatctgcgcagccgccatgccggggttttacgagattgtgattaaggtccccagcgaccttgacgagcatctgcccggcatttctgacagctttgtgaactgggtggccgagaaggaatgggagttgccgccagattctgacatggatctgaatctgattgagcaggcacccctgaccgtggccgagaagctgcagcgcgactttctgacggaatggcgccgtgtgagtaaggccccggaggcccttttctttgtgcaatttgagaagggagagagctacttccacatgcacgtgctcgtggaaaccaccggggtgaaatccatggttttgggacgtttcctgagtcagattcgcgaaaaactgattcagagaatttaccgcgggatcgagccgactttgccaaactggttcgcggtcacaaagaccagaaatggcgccggaggcgggaacaaggtggtggatgagtgctacatccccaattacttgctccccaaaacccagcctgagctccagtgggcgtggactaatatggaacagtatttaagcgcctgtttgaatctcacggagcgtaaacggttggtggcgcagcatctgacgcacgtgtcgcagacgcaggagcagaacaaagagaatcagaatcccaattctgatgcgccggtgatcagatcaaaaacttcagccaggtacatggagctggtcgggtggctcgtggacaaggggattacctcggagaagcagtggatccaggaggaccaggcctcatacatctccttcaatgcggcctccaactcgcggtcccaaatcaaggctgccttggacaatgcgggaaagattatgagcctgactaaaaccgcccccgactacctggtgggccagcagcccgtggaggacatttccagcaatcggatttataaaattttggaactaaacgggtacgatccccaatatgcggcttccgtctttctgggatgggccacgaaaaagttcggcaagaggaacaccatctggctgtttgggcctgcaactaccgggaagaccaacatcgcggaggccatagcccacactgtgcccttctacgggtgcgtaaactggaccaatgagaactttcccttcaacgactgtgtcgacaagatggtgatctggtgggaggaggggaagatgaccgccaaggtcgtggagtcggccaaagccattctcggaggaagcaaggtgcgcgtggaccagaaatgcaagtcctcggcccagatagacccgactcccgtgatcgtcacctccaacaccaacatgtgcgccgtgattgacgggaactcaacgaccttcgaacaccagcagccgttgcaagaccggatgttcaaatttgaactcacccgccgtctggatcatgactttgggaaggtcaccaagcaggaagtcaaagactttttccggtgggcaaaggatcacgtggttgaggtggagcatgaattctacgtcaaaaagggtggagccaagaaaagacccgcccccagtgacgcagatataagtgagcccaaacgggtgcgcgagtcagttgcgcagccatcgacgtcagacgcggaagcttcgatcaactacgcagacaggtaccaaaacaaatgttctcgtcacgtgggcatgaatctgatgctgtttccctgcagacaatgcgagagaatgaatcagaattcaaatatctgcttcactcacggacagaaagactgtttagagtgctttcccgtgtcagaatctcaacccgtttctgtcgtcaaaaaggcgtatcagaaactgtgctacattcatcatatcatgggaaaggtgccagacgcttgcactgcctgcgatctggtcaatgtggatttggatgactgcatctttgaacaataaatgatttaaatcaggtatgtcttttgttgatcaccctccagattggttggaagaagttggtgaaggtcttcgcgagtttttgggccttgaagcgggcccaccgaaaccaaaacccaatcagcagcatcaagatcaagcccgtggtcttgtgctgcctggttataactatctcggacccggaaacggtctcgatcgaggagagcctgtcaacagggcagacgaggtcgcgcgagagcacgacatctcgtacaacgagcagcttgaggcgggagacaacccctacctcaagtacaaccacgcggacgccgagtttcaggagaagctcgccgacgacacatccttcgggggaaacctcggaaaggcagtctttcaggccaagaaaagggttctcgaaccttttggcctggttgaagagggtgctaagacggcccctaccggaaagcggatagacgaccactttccaaaaagaaagaaggctcggaccgaagaggactccaagccttccacctcgtcagacgccgaagctggacccagcggatcccagcagctgcaaatcccagcccaaccagcctcaagtttgggagctgatacaatgtctgcgggaggtggcggcccattgggcgacaataaccaaggtgccgatggagtgggcaatgcctcgggagattggcattgcgattccacgtggatgggggacagagtcgtcaccaagtccacccgaacctgggtgctgcccagctacaacaaccaccagtaccgagagatcaaaagcggctccgtcgacggaagcaacgccaacgcctactttggatacagcaccccctgggggtactttgactttaaccgcttccacagccactggagcccccgagactggcaaagactcatcaacaactactggggcttcagaccccggtccctcagagtcaaaatcttcaacattcaagtcaaagaggtcacggtgcaggactccaccaccaccatcgccaacaacctcacctccaccgtccaagtgtttacggacgacgactaccagctgccctacgtcgtcggcaacgggaccgagggatgcctgccggccttccctccgcaggtctttacgctgccgcagtacggttacgcgacgctgaaccgcgacaacacagaaaatcccaccgagaggagcagcttcttctgcctagagtactttcccagcaagatgctgagaacgggcaacaactttgagtttacctacaactttgaggaggtgcccttccactccagcttcgctcccagtcagaacctgttcaagctggccaacccgctggtggaccagtacttgtaccgcttcgtgagcacaaataacactggcggagtccagttcaacaagaacctggccgggagatacgccaacacctacaaaaactggttcccggggcccatgggccgaacccagggctggaacctgggctccggggtcaaccgcgccagtgtcagcgccttcgccacgaccaataggatggagctcgagggcgcgagttaccaggtgcccccgcagccgaacggcatgaccaacaacctccagggcagcaacacctatgccctggagaacactatgatcttcaacagccagccggcgaacccgggcaccaccgccacgtacctcgagggcaacatgctcatcaccagcgagagcgagacgcagccggtgaaccgcgtggcgtacaacgtcggcgggcagatggccaccaacaaccagagctccaccactgcccccgcgaccggcacgtacaacctccaggaaatcgtgcccggcagcgtgtggatggagagggacgtgtacctccaaggacccatctgggccaagatcccagagacgggggcgcactttcacccctctccggccatgggcggattcggactcaaacacccaccgcccatgatgctcatcaagaacacgcctgtgcccggaaatatcaccagcttctcggacgtgcccgtcagcagcttcatcacccagtacagcaccgggcaggtcaccgtggagatggagtgggagctcaagaaggaaaactccaagaggtggaacccagagatccagtacacaaacaactacaacgacccccagtttgtggactttgccccggacagcaccggggaatacagaaccaccagacctatcggaacccgataccttacccgacccctttaattgcttgttaatcaataaaccgtttaattcgtttcagttgaactttggtctctgcgtatttctttcttatctagtttccatggctacgtagataagtagcatggcgggttaatcattaactacagcccgggcgtttaaacagcgggcggaggggtggagtcgtgacgtgaattacgtcatagggttagggaggtcctgtattagaggtcacgtgagtgttttgcgacattttgcgacaccatgtggtctcgctgggggggggggcccgagtgagcacgcagggtctccattttgaagcgggaggtttgaacgagcgctggcgcgctcactggccgtcgttttacaacgtcgtgactgggaaaaccctggcgttacccaacttaatcgccttgcagcacatccccctttcgccagctggcgtaatagcgaagaggcccgcaccgatcgcccttcccaacagttgcgcagcctgaatggcgaatggaaattgtaagcgttaatattttgttaaaattcgcgttaaatttttgttaaatcagctcatttttttaaccaataggccgaaatcggcaaaatcccttataaatcaaaagaatagaccgagatagggttgagtgttgttccagtttggaacaagagtccactattaagaacgtggactccaacgtcaaagggcgaaaaaccgtctatcagggcgatggcccactacgtgaaccatcaccctaatcaagttttttggggtcgaggtgccgtaaagcactaaatcggaaccctaaagggagcccccgatttagagcttgacggggaaagccggcgaacgtggcgagaaaggaagggaagaaagcgaaaggagcgggcgctagggcgctggcaagtgtagcggtcacgctgcgcgtaaccaccacacccgccgcgcttaatgcgccgctacagggcgcgtcaggtggcacttttcggggaaatgtgcgcggaacccctatttgtttatttttctaaatacattcaaatatgtatccgctcatgagacaataaccctgataaatgcttcaataatattgaaaaaggaagagtatgagtattcaacatttccgtgtcgcccttattcccttttttgcggcattttgccttcctgtttttgctcacccagaaacgctggtgaaagtaaaagatgctgaagatcagttgggtgcacgagtgggttacatcgaactggatctcaacagcggtaagatccttgagagttttcgccccgaagaacgttttccaatgatgagcacttttaaagttctgctatgtggcgcggtattatcccgtattgacgccgggcaagagcaactcggtcgccgcatacactattctcagaatgacttggttgagtactcaccagtcacagaaaagcatcttacggatggcatgacagtaagagaattatgcagtgctgccataaccatgagtgataacactgcggccaacttacttctgacaacgatcggaggaccgaaggagctaaccgcttttttgcacaacatgggggatcatgtaactcgccttgatcgttgggaaccggagctgaatgaagccataccaaacgacgagcgtgacaccacgatgcctgtagcaatggcaacaacgttgcgcaaactattaactggcgaactacttactctagcttcccggcaacaattaatagactggatggaggcggataaagttgcaggaccacttctgcgctcggcccttccggctggctggtttattgctgataaatctggagccggtgagcgtgggtctcgcggtatcattgcagcactggggccagatggtaagccctcccgtatcgtagttatctacacgacggggagtcaggcaactatggatgaacgaaatagacagatcgctgagataggtgcctcactgattaagcattggtaactgtcagaccaagtttactcatatatactttagattgatttaaaacttcatttttaatttaaaaggatctaggtgaagatcctttttgataatctcatgaccaaaatcccttaacgtgagttttcgttccactgagcgtcagaccccgtagaaaagatcaaaggatcttcttgagatcctttttttctgcgcgtaatctgctgcttgcaaacaaaaaaaccaccgctaccagcggtggtttgtttgccggatcaagagctaccaactctttttccgaaggtaactggcttcagcagagcgcagataccaaatactgttcttctagtgtagccgtagttaggccaccacttcaagaactctgtagcaccgcctacatacctcgctctgctaatcctgttaccagtggctgctgccagtggcgataagtcgtgtcttaccgggttggactcaagacgatagttaccggataaggcgcagcggtcgggctgaacggggggttcgtgcacacagcccagcttggagcgaacgacctacaccgaactgagatacctacagcgtgagctatgagaaagcgccacgcttcccgaagggagaaaggcggacaggtatccggtaagcggcagggtcggaacaggagagcgcacgagggagcttccagggggaaacgcctggtatctttatagtcctgtcgggtttcgccacctctgacttgagcgtcgatttttgtgatgctcgtcaggggggcggagcctatggaaaaacgccagcaacgcggcctttttacggttcctggccttttgctggccttttgctcacatgttctttcctgcgttatcccctgattctgtggataaccgtattaccgcctttgagtgagctgataccgctcgccgcagccgaacgaccgagcgcagcgagtcagtgagcgaggaagcggaagagcgcccaatacgcaaaccgcctctccccgcgcgttggccgattcattaatgcagctggcacgacaggtttcccgactggaaagcgggcagtgagcgcaacgcaattaatgtgagttagctcactcattaggcaccccaggctttacactttatgcttccggctcgtatgttgtgtggaattgtgagcggataacaatttcacacaggaaacagctatgaccatgattacgccaa

SEQ ID NO: 3 - DNA, 11635 bp, synthetic construct
  misc_feature 1..11635: note = plasmid
  source 1..11635: mol_type = other DNA
ggtacccaactccatgcttaacagtccccaggtacagcccaccctgcgtcgcaaccaggaacagctctacagcttcctggagcgccactcgccctacttccgcagccacagtgcgcagattaggagcgccacttctttttgtcacttgaaaaacatgtaaaaataatgtactaggagacactttcaataaaggcaaatgtttttatttgtacactctcgggtgattatttaccccccacccttgccgtctgcgccgtttaaaaatcaaaggggttctgccgcgcatcgctatgcgccactggcagggacacgttgcgatactggtgtttagtgctccacttaaactcaggcacaaccatccgcggcagctcggtgaagttttcactccacaggctgcgcaccatcaccaacgcgtttagcaggtcgggcgccgatatcttgaagtcgcagttggggcctccgccctgcgcgcgcgagttgcgatacacagggttgcagcactggaacactatcagcgccgggtggtgcacgctggccagcacgctcttgtcggagatcagatccgcgtccaggtcctccgcgttgctcagggcgaacggagtcaactttggtagctgccttcccaaaaagggtgcatgcccaggctttgagttgcactcgcaccgtagtggcatcagaaggtgaccgtgcccggtctgggcgttaggatacagcgcctgcatgaaagccttgatctgcttaaaagccacctgagcctttgcgccttcagagaagaacatgccgcaagacttgccggaaaactgattggccggacaggccgcgtcatgcacgcagcaccttgcgtcggtgttggagatctgcaccacatttcggccccaccggttcttcacgatcttggccttgctagactgctccttcagcgcgcgctgcccgttttcgctcgtcacatccatttcaatcacgtgctccttatttatcataatgctcccgtgtagacacttaagctcgccttcgatctcagcgcagcggtgcagccacaacgcgcagcccgtgggctcgtggtgcttgtaggttacctctgcaaacgactgcaggtacgcctgcaggaatcgccccatcatcgtcacaaaggtcttgttgctggtgaaggtcagctgcaacccgcggtgctcctcgtttagccaggtcttgcatacggccgccagagcttccacttggtcaggcagtagcttgaagtttgcctttagatcgttatccacgtggtacttgtccatcaacgcgcgcgcagcctccatgcccttctcccacgcagacacgatcggcaggctcagcgggtttatcaccgtgctttcactttccgcttcactggactcttccttttcctcttgcgtccgcataccccgcgccactgggtcgtcttcattcagccgccgcaccgtgcgcttacctcccttgccgtgcttgattagcaccggtgggttgctgaaacccaccatttgtagcgccacatcttctctttcttcctcgctgtccacgatcacctctggggatggcgggcgctcgggcttgggagaggggcgcttctttttctttttggacgcaatggccaaatccgccgtcgaggtcgatggccgcgggctgggtgtgcgcggcaccagcgcatcttgtgacgagtcttcttcgtcctcggactcgagacgccgcctcagccgcttttttgggggcgcgcggggaggcggcggcgacggcgacggggacgacacgtcctccatggttggtggacgtcgcgccgcaccgcgtccgcgctcgggggtggtttcgcgctgctcctcttcccgactggccatttccttctcctataggcagaaaaagatcatggagtcagtcgagaaggaggacagcctaaccgccccctttgagttcgccaccaccgcctccaccgatgccgccaacgcgcctaccaccttccccgtcgaggcacccccgcttgaggaggaggaagtgattatcgagcaggacccaggttttgtaagcgaagacgacgaggatcgctcagtaccaacagaggataaaaagcaagaccaggacgacgcagaggcaaacgaggaacaagtcgggcggggggaccaaaggcatggcgactacctagatgtgggagacgacgtgctgttgaagcatctgcagcgccagtgcgccattatctgcgacgcgttgcaagagcgcagcgatgtgcccctcgccatagcggatgtcagccttgcctacgaacgccacctgttctcaccgcgcgtaccccccaaacgccaagaaaacggcacatgcgagcccaacccgcgcctcaacttctaccccgtatttgccgtgccagaggtgcttgccacctatcacatctttttccaaaactgcaagatacccctatcctgccgtgccaaccgcagccgagcggacaagcagctggccttgcggcagggcgctgtcatacctgatatcgcctcgctcgacgaagtgccaaaaatctttgagggtcttggacgcgacgagaaacgcgcggcaaacgctctgcaacaagaaaacagcgaaaatgaaagtcactgtggagtgctggtggaacttgagggtgacaacgcgcgcctagccgtgctgaaacgcagcatcgaggtcacccactttgcctacccggcacttaacctaccccccaaggttatgagcacagtcatgagcgagctgatcgtgcgccgtgcacgacccctggagagggatgcaaacttgcaagaacaaaccgaggagggcctacccgcagttggcgatgagcagctggcgcgctggcttgagacgcgcgagcctgccgacttggaggagcgacgcaagctaatgatggccgcagtgcttgttaccgtggagcttgagtgcatgcagcggttctttgctgacccggagatgcagcgcaagctagaggaaacgttgcactacacctttcgccagggctacgtgcgccaggcctgcaaaatttccaacgtggagctctgcaacctggtctcctaccttggaattttgcacgaaaaccgcctcgggcaaaacgtgcttcattccacgctcaagggcgaggcgcgccgcgactacgtccgcgactgcgtttacttatttctgtgctacacctggcaaacggccatgggcgtgtggcagcaatgcctggaggagcgcaacctaaaggagctgcagaagctgctaaagcaaaacttgaaggacctatggacggccttcaacgagcgctccgtggccgcgcacctggcggacattatcttccccgaacgcctgcttaaaaccctgcaacagggtctgccagacttcaccagtcaaagcatgttgcaaaactttaggaactttatcctagagcgttcaggaattctgcccgccacctgctgtgcgcttcctagcgactttgtgcccattaagtaccgtgaatgccctccgccgctttggggtcactgctaccttctgcagctagccaactaccttgcctaccactccgacatcatggaagacgtgagcggtgacggcctactggagtgtcactgtcgctgcaacctatgcaccccgcaccgctccctggtctgcaattcgcaactgcttagcgaaagtcaaattatcggtacctttgagctgcagggtccctcgcctgacgaaaagtccgcggctccggggttgaaactcactccggggctgtggacgtcggcttaccttcgcaaatttgtacctgaggactaccacgcccacgagattaggttctacgaagaccaatcccgcccgccaaatgcggagcttaccgcctgcgtcattacccagggccacatccttggccaattgcaagccatcaacaaagcccgccaagagtttctgctacgaaagggacggggggtttacctggacccccagtccggcgaggagctcaacccaatccccccgccgccgcagccctatcagcagccgcgggcccttgcttcccaggatggcacccaaaaagaagctgcagctgccgccgccgccacccacggacgaggaggaatactgggacagtcaggcagaggaggttttggacgaggaggaggagatgatggaagactgggacagcctagacgaagcttccgaggccgaagaggtgtcagacgaaacaccgtcaccctcggtcgcattcccctcgccggcgccccagaaattggcaaccgttcccagcatcgctacaacctccgctcctcaggcgccgccggcactgcctgttcgccgacccaaccgtagatgggacaccactggaaccagggccggtaagtctaagcagccgccgccgttagcccaagagcaacaacagcgccaaggctaccgctcgtggcgcgggcacaagaacgccatagttgcttgcttgcaagactgtgggggcaacatctccttcgcccgccgctttcttctctaccatcacggcgtggccttcccccgtaacatcctgcattactaccgtcatctctacagcccctactgcaccggcggcagcggcagcggcagcaacagcagcggtcacacagaagcaaaggcgaccggatagcaagactctgacaaagcccaagaaatccacagcggcggcagcagcaggaggaggagcgctgcgtctggcgcccaacgaacccgtatcgacccgcgagcttagaaataggatttttcccactctgtatgctatatttcaacaaagcaggggccaagaacaagagctgaaaataaaaaacaggtctctgcgctccctcacccgcagctgcctgtatcacaaaagcgaagatcagcttcggcgcacgctggaagacgcggaggctctcttcagcaaatactgcgcgctgactcttaaggactagtttcgcgccctttctcaaatttaagcgcgaaaactacgtcatctccagcggccacacccggcgccagcacctgtcgtcagcgccattatgagcaaggaaattcccacgccctacatgtggagttaccagccacaaatgggacttgcggctggagctgcccaagactactcaacccgaataaactacatgagcgcgggaccccacatgatatcccgggtcaacggaatccgcgcccaccgaaaccgaattctcctcgaacaggcggctattaccaccacacctcgtaataaccttaatccccgtagttggcccgctgccctggtgtaccaggaaagtcccgctcccaccactgtggtacttcccagagacgcccaggccgaagttcagatgactaactcaggggcgcagcttgcgggcggctttcgtcacagggtgcggtcgcccgggcgttttagggcggagtaacttgcatgtattgggaattgtagtttttttaaaatgggaagtgacgtatcgtgggaaaacggaagtgaagatttgaggaagttgtgggttttttggctttcgtttctgggcgtaggttcgcgtgcggttttctgggtgttttttgtggactttaaccgttacgtcattttttagtcctatatatactcgctctgtacttggccctttttacactgtgactgattgagctggtgccgtgtcgagtggtgttttttaataggtttttttactggtaaggctgactgttatggctgccgctgtggaagcgctgtatgttgttctggagcgggagggtgctattttgcctaggcaggagggtttttcaggtgtttatgtgtttttctctcctattaattttgttatacctcctatgggggctgtaatgttgtctctacgcctgcgggtatgtattcccccgggctatttcggtcgctttttagcactgaccgatgttaaccaacctgatgtgtttaccgagtcttacattatgactccggacatgaccgaggaactgtcggtggtgctttttaatcacggtgaccagtttttttacggtcacgccggcatggccgtagtccgtcttatgcttataagggttgtttttcctgttgtaagacaggcttctaatgtttaaatgtttttttttttgttattttattttgtgtttaatgcaggaacccgcagacatgtttgagagaaaaatggtgtctttttctgtggtggttccggaacttacctgcctttatctgcatgagcatgactacgatgtgcttgcttttttgcgcgaggctttgcctgattttttgagcagcaccttgcattttatatcgccgcccatgcaacaagcttacataggggctacgctggttagcatagctccgagtatgcgtgtcataatcagtgtgggttcttttgtcatggttcctggcggggaagtggccgcgctggtccgtgcagacctgcacgattatgttcagctggccctgcgaagggacctacgggatcgcggtatttttgttaatgttccgcttttgaatcttatacaggtctgtgaggaacctgaatttttgcaatcatgattcgctgcttgaggctgaaggtggagggcgctctggagcagatttttacaatggccggacttaatattcgggatttgcttagagacatattgataaggtggcgagatgaaaattatttgggcatggttgaaggtgctggaatgtttatagaggagattcaccctgaagggtttagcctttacgtccacttggacgtgagggcagtttgccttttggaagccattgtgcaacatcttacaaatgccattatctgttctttggctgtagagtttgaccacgccaccggaggggagcgcgttcacttaatagatcttcattttgaggttttggataatcttttggaataaaaaaaaaaaaacatggttcttccagctcttcccgctcctcccgtgtgtgactcgcagaacgaatgtgtaggttggctgggtgtggcttattctgcggtggtggatgttatcagggcagcggcgcatgaaggagtttacatagaacccgaagccagggggcgcctggatgctttgagagagtggatatactacaactactacacagagcgagctaagcgacgagaccggagacgcagatctgtttgtcacgcccgcacctggttttgcttcaggaaatatgactacgtccggcgttccatttggcatgacactacgaccaacacgatctcggttgtctcggcgcactccgtacagtagggatcgcctacctccttttgagacagagacccgcgctaccatactggaggatcatccgctgctgcccgaatgtaacactttgacaatgcacaacgtgagttacgtgcgaggtcttccctgcagtgtgggatttacgctgattcaggaatgggttgttccctgggatatggttctgacgcgggaggagcttgtaatcctgaggaagtgtatgcacgtgtgcctgtgttgtgccaacattgatatcatgacgagcatgatgatccatggttacgagtcctgggctctccactgtcattgttccagtcccggttccctgcagtgcatagccggcgggcaggttttggccagctggtttaggatggtggtggatggcgccatgtttaatcagaggtttatatggtaccgggaggtggtgaattacaacatgccaaaagaggtaatgtttatgtccagcgtgtttatgaggggtcgccacttaatctacctgcgcttgtggtatgatggccacgtgggttctgtggtccccgccatgagctttggatacagcgccttgcactgtgggattttgaacaatattgtggtgctgtgctgcagttactgtgctgatttaagtgagatcagggtgcgctgctgtgcccggaggacaaggcgtctcatgctgcgggcggtgcgaatcatcgctgaggagaccactgccatgttgtattcctgcaggacggagcggcggcggcagcagtttattcgcgcgctgctgcagcaccaccgccctatcctgatgcacgattatgactctacccccatgtaggcgtggacttccccttcgccgcccgttgagcaaccgcaagttggacagcagcctgtggctcagcagctggacagcgacatgaacttaagcgagctgcccggggagtttattaatatcactgatgagcgtttggctcgacaggaaaccgtgtggaatataacacctaagaatatgtctgttacccatgatatgatgctttttaaggccagccggggagaaaggactgtgtactctgtgtgttgggagggaggtggcaggttgaatactagggttctgtgagtttgattaaggtacggtgatcaatataagctatgtggtggtggggctatactactgaatgaaaaatgacttgaaattttctgcaattgaaaaataaacacgttgaaacataacatgcaacaggttcacgattctttattcctgggcaatgtaggagaaggtgtaagagttggtagcaaaagtttcagtggtgtattttccactttcccaggaccatgtaaaagacatagagtaagtgcttacctcgctagtttctgtggattcactagaatcgatgtaggatgttgcccctcctgacgcggtaggagaaggggagggtgccctgcatgtctgccgctgctcttgctcttgccgctgctgaggaggggggcgcatctgccgcagcaccggatgcatctgggaaaagcaaaaaaggggctcgtccctgtttccggaggaatttgcaagcggggtcttgcatgacggggaggcaaacccccgttcgccgcagtccggccggcccgagactcgaaccgggggtcctgcgactcaacccttggaaaataaccctccggctacagggagcgagccacttaatgctttcgctttccagcctaaccgcttacgccgcgcgcggccagtggccaaaaaagctagcgcagcagccgccgcgcctggaaggaagccaaaaggagcgctcccccgttgtctgacgtcgcacacctgggttcgacacgcgggcggtaaccgcatggatcacggcggacggccggatccggggttcgaaccccggtcgtccgccatgatacccttgcgaatttatccaccagaccacggaagagtgcccgcttacaggctctccttttgcacggtctagagcgtcaacgactgcgcacgcctcaccggccagagcgtcccgaccatggagcactttttgccgctgcgcaacatctggaaccgcgtccgcgactttccgcgcgcctccaccaccgccgccggcatcacctggatgtccaggtacatctacggattacgtcgacgtttaaaccatatgatcagctcactcaaaggcggtaatacggttatccacagaatcaggggataacgcaggaaagaacatgtgagcaaaaggccagcaaaaggccaggaaccgtaaaaaggccgcgttgctggcgtttttccataggctccgcccccctgacgagcatcacaaaaatcgacgctcaagtcagaggtggcgaaacccgacaggactataaagataccaggcgtttccccctggaagctccctcgtgcgctctcctgttccgaccctgccgcttaccggatacctgtccgcctttctcccttcgggaagcgtggcgctttctcatagctcacgctgtaggtatctcagttcggtgtaggtcgttcgctccaagctgggctgtgtgcacgaaccccccgttcagcccgaccgctgcgccttatccggtaactatcgtcttgagtccaacccggtaagacacgacttatcgccactggcagcagccactggtaacaggattagcagagcgaggtatgtaggcggtgctacagagttcttgaagtggtggcctaactacggctacactagaagaacagtatttggtatctgcgctctgctgaagccagttaccttcggaaaaagagttggtagctcttgatccggcaaacaaaccaccgctggtagcggtggtttttttgtttgcaagcagcagattacgcgcagaaaaaaaggatctcaagaagatcctttgatcttttctacggggtctgacgctcagtggaacgaaaactcacgttaagggattttggtcatgagattatcaaaaaggatcttcacctagatccttttaaattaaaaatgaagttttaaatcaatctaaagtatatatgagtaaacttggtctgacagttaccaatgcttaatcagtgaggcacctatctcagcgatctgtctatttcgttcatccatagttgcctgactccccgtcgtgtagataactacgatacgggagggcttaccatctggccccagtgctgcaatgataccgcgagacccacgctcaccggctccagatttatcagcaataaaccagccagccggaagggccgagcgcagaagtggtcctgcaactttatccgcctccatccagtctattaattgttgccgggaagctagagtaagtagttcgccagttaatagtttgcgcaacgttgttgccattgctacaggcatcgtggtgtcacgctcgtcgtttggtatggcttcattcagctccggttcccaacgatcaaggcgagttacatgatcccccatgttgtgcaaaaaagcggttagctccttcggtcctccgatcgttgtcagaagtaagttggccgcagtgttatcactcatggttatggcagcactgcataattctcttactgtcatgccatccgtaagatgcttttctgtgactggtgagtactcaaccaagtcattctgagaatagtgtatgcggcgaccgagttgctcttgcccggcgtcaatacgggataataccgcgccacatagcagaactttaaaagtgctcatcattggaaaacgttcttcggggcgaaaactctcaaggatcttaccgctgttgagatccagttcgatgtaacccactcgtgcacccaactgatcttcagcatcttttactttcaccagcgtttctgggtgagcaaaaacaggaaggcaaaatgccgcaaaaaagggaataagggcgacacggaaatgttgaatactcatactcttcctttttcaatattattgaagcatttatcagggttattgtctcatgagcggatacatatttgaatgtatttagaaaaataaacaaataggggttccgcgcacatttccccgaaaagtgccacctaaattgtaagcgttaatattttgttaaaattcgcgttaaatttttgttaaatcagctcattttttaaccaataggccgaaatcggcaaaatcccttataaatcaaaagaatagaccgagatagggttgagtgttgttccagtttggaacaagagtccactattaaagaacgtggactccaacgtcaaagggcgaaaaaccgtctatcagggcgatggcccactacgtgaaccatcaccctaatcaagttttttggggtcgaggtgccgtaaagcactaaatcggaaccctaaagggagcccccgatttagagcttgacggggaaagccggcgaacgtggcgagaaaggaagggaagaaagcgaaaggagcgggcgctagggcgctggcaagtgtagcggtcacgctgcgcgtaaccaccacacccgccgcgcttaatgcgccgctacagggcgcgatggatcc